European Patent Application EP 4 119 167 A1, published January 18, 2023. Title: A single-stranded nucleic acids and a composition for inducing -1 frameshift. Applicant: YANO, Takamitsu. The sequence listing filed with the application follows.

SEQUENCE LISTING (18 sequences)

SEQ ID NO: 1 - RNA, 38 nt, Artificial sequence
  Artificial RNA
cgcugccguccccgcauuacccccccccccuagugugg

SEQ ID NO: 2 - RNA, 39 nt, Artificial sequence
  Artificial RNA
ccgauugauuccgcgcauuacccccccccccuagugugc

SEQ ID NO: 3 - RNA, 38 nt, Artificial sequence
  Artificial RNA
guaacagucuggcgcauuacccccccccccuagugugc

SEQ ID NO: 4 - RNA, 39 nt, Artificial sequence
  Artificial RNA
cugaguaggagcccgcauuacccccccccccuagugugg

SEQ ID NO: 5 - RNA, 39 nt, Artificial sequence
  Artificial RNA
uaccauuuguaugcgcauuacccccccccccuagugugc

SEQ ID NO: 6 - RNA, 38 nt, Artificial sequence
  Artificial RNA
cgaugccggugccgcauuacccccccccccuagugugg

SEQ ID NO: 7 - DNA, 717 bp, Artificial sequence
  Artificial DNA
atggtgagcaagggcgaggagctgttcaccggggtggtgcccatcctggtcgagctggacggcgacgtaaacggccacaagttcagcgtgtccggcgagggcgagggcgatgccacctacggcaagctgaccctgaagttcatctgcaccaccggcaagctgcccgtgccctggcccaccctcgtgaccaccctgacctacggcgtgcagtgcttcagccgctaccccgaccacatgaagcagcacgacttcttcaagtccgccatgcccgaaggctacgtccaggagcgcaccatcttcttcaaggacgacggcaactacaagacccgcgccgaggtgaagttcgagggcgacaccctggtgaaccgcatcgagctgaagggcatcgacttcaaggaggacggcaacatcctggggcacaagctggagtacaactacaacagccacaacgtctatatcatggccgacaagcagaagaacggcatcaaggtgaacttcaagatccgccacaacatcgaggacggcagcgtgcagctcgccgaccactaccagcagaacacccccatcggcgacggccccgtgctgctgcccgacaaccactacctgagcacccagtccgccctgagcaaagaccccaacgagaagcgcgatcacatggtcctgctggagttcgtgaccgccgccgggatcactctcggcatggacgagctgtacaag

SEQ ID NO: 8 - DNA, 18 bp, Artificial sequence
  Artificial DNA
tccggactcagatctcga

SEQ ID NO: 9 - DNA, 1356 bp, Homo sapiens
gtgcgtgagtgcatctccatccacgttggccaggctggtgtccagattggcaatgcctgctgggagctctactgcctggaacacggcatccagcccgatggccagatgccaagtgacaagaccattgggggaggagatgactccttcaacaccttcttcagtgagacgggcgctggcaagcacgtgccccgggctgtgtttgtagacttggaacccacagtcattgatgaagttcgcactggcacctaccgccagctcttccaccctgagcagctcatcacaggcaaggaagatgctgccaataactatgcccgagggcactacaccattggcaaggagatcattgaccttgtgttggaccgaattcgcaagctggctgaccagtgcaccggtcttcagggcttcttggttttccacagctttggtgggggaactggttctgggttcacctccctgctcatggaacgtctctcagttgattatggcaagaagtccaagctggagttctccatttacccagcaccccaggtttccacagctgtagttgagccctacaactccatcctcaccacccacaccaccctggagcactctgattgtgccttcatggtagacaatgaggccatctatgacatctgtcgtagaaacctcgatatcgagcgcccaacctacactaaccttaaccgccttattagccagattgtgtcctccatcactgcttccctgagatttgatggagccctgaatgttgacctgacagaattccagaccaacctggtgccctacccccgcatccacttccctctggccacatatgcccctgtcatctctgctgagaaagcctaccatgaacagctttctgtagcagagatcaccaatgcttgctttgagccagccaaccagatggtgaaatgtgaccctcgccatggtaaatacatggcttgctgcctgttgtaccgtggtgacgtggttcccaaagatgtcaatgctgccattgccaccatcaaaaccaagcgcagcatccagtttgtggattggtgccccactggcttcaaggttggcatcaactaccagcctcccactgtggtgcctggtggagacctggccaaggtacagagagctgtgtgcatgctgagcaacaccacagccattgctgaggcctgggctcgcctggaccacaagtttgacctgatgtatgccaagcgtgcctttgttcactggtacgtgggtgaggggatggaggaaggcgagttttcagaggcccgtgaagatatggctgcccttgagaaggattatgaggaggttggtgtggattctgttgaaggagagggtgaggaagaaggagaggaatactaa

SEQ ID NO: 10 - DNA, 480 bp, Escherichia coli
atgatcagtctgattgcggcgttagcggtagatcgcgttatcggcatggaaaacgccatgccgtggaacctgcctgccgatctcgcctggtttaaacgcaacaccttaaataaacccgtgattatgggccgccatacctgggaatcaatcggtcgtccgttgccaggacgcaaaaatattatcctcagcagtcaaccgggtacggacgatcgcgtaacgtgggtgaagtcggtggatgaagccatcgcggcgtgtggtgacgtaccagaaatcatggtgattggcggcggtcgcgtttatgaacagttcttgccaaaagcgcaaaaactgtatctgacgcatatcgacgcagaagtggaaggcgacacccatttcccggattacgagccggatgactgggaatcggtattcagcgaattccacgatgctgatgcgcagaactctcacagctattgctttgagattctggagcggcggtaa

SEQ ID NO: 11 - DNA, 16 bp, Artificial sequence
  Primer
gaaattaatacgactc

SEQ ID NO: 12 - DNA, 50 bp, Artificial sequence
  Primer
atccatttaattagtggtgatggtgatgatgtccaccgacttcacccacg

SEQ ID NO: 13 - protein, 159 aa, Escherichia coli [sequence omitted]

SEQ ID NO: 14 - protein, 85 aa, Artificial sequence
  Artificial protein
MISLIAALAVDRVIGMENAMPWNLPADLAWFKRNTLNKPVIMGRPYLGINRSSVARTQKYYPQQSTGYGRSRNVGEVGGHHHHHH

SEQ ID NO: 15 - RNA, 8 nt, Artificial sequence
  Artificial RNA
ccgcauua

SEQ ID NO: 16 - RNA, 8 nt, Artificial sequence
  Artificial RNA
uagugugg

SEQ ID NO: 17 - RNA, 27 nt, Artificial sequence
  Artificial RNA
ccgcauuacccccccccccuagugugg

SEQ ID NO: 18 - RNA, 27 nt, Artificial sequence
  Artificial RNA
gcgcauuacccccccccccuagugugc